European Patent Application EP 4 438 055 A1, published October 2, 2024. Title: ANTI-SIGLEC-15 ANTIBODY AND USE THEREOF. Applicant: CHIA TAI TIANQING PHARMACEUTICAL GROUP CO., LTD. Application EP 22897899.5, filed November 24, 2022. The sequence listing filed with the application follows.

SEQUENCE LISTING (156 sequences)

SEQ ID NO: 1 - protein, 328 aa, Homo sapiens
MEKSIWLLACLAWVLPTGSFVRTKIDTTENLLNTEVHSSPAQRWSMQVPPEVSAEAGDAAVLPCTFTHPHRHYDGPLTAIWRAGEPYAGPQVFRCAAARGSELCQTALSLHGRFRLLGNPRRNDLSLRVERLALADDRRYFCRVEFAGDVHDRYESRHGVRLHVTAAPRIVNISVLPSPAHAFRALCTAEGEPPPALAWSGPALGNSLAAVRSPREGHGHLVTAELPALTHDGRYTCTAANSLGRSEASVYLFRFHGASGASTVALLLGALGFKALLLLGVLAARAARRRPEHLDTPDTPPRSQAQESNYENLSQMNPRSPPATMCSP

SEQ ID NO: 2 - protein, 454 aa, synthetic construct
  REGION 1..454: note = PR300526 H
  source 1..454: note = PR300526 H
QVQLVQSGAEVKKPGASVKVSCKASGYTFTDYYMHWVRQAPGQGLEWMGWINPNSDGTNYAQRFQGRVTMTRDTSISTAYMELSRLRSDDTAVYYCARGRLLRFFDWLDVMDAWGQGTSVTVSSASTKGPSVFPLAPSSKSTSGGTAALGCLVKDYFPEPVTVSWNSGALTSGVHTFPAVLQSSGLYSLSSVVTVPSSSLGTQTYICNVNHKPSNTKVDKKVEPKSCDKTHTCPPCPAPELLGGPSVFLFPPKPKDTLMISRTPEVTCVVVDVSHEDPEVKFNWYVDGVEVHNAKTKPREEQYNSTYRVVSVLTVLHQDWLNGKEYKCKVSNKALPAPIEKTISKAKGQPREPQVYTLPPSREEMTKNQVSLTCLVKGFYPSDIAVEWESNGQPENNYKTTPPVLDSDGSFFLYSKLTVDKSRWQQGNVFSCSVMHEALHNHYTQKSLSLSPGK

SEQ ID NO: 3 - protein, 124 aa, synthetic construct
  REGION 1..124: note = PR300526 VH
  source 1..124: note = PR300526 VH
QVQLVQSGAEVKKPGASVKVSCKASGYTFTDYYMHWVRQAPGQGLEWMGWINPNSDGTNYAQRFQGRVTMTRDTSISTAYMELSRLRSDDTAVYYCARGRLLRFFDWLDVMDAWGQGTSVTVSS

SEQ ID NO: 4 - protein, 25 aa, synthetic construct [sequence omitted]

SEQ ID NO: 5 - protein, 10 aa, synthetic construct
  REGION 1..10: note = PR300526 HCDR1
  source 1..10: note = PR300526 HCDR1
GYTFTDYYMH

SEQ ID NO: 6 - protein, 14 aa, synthetic construct
  REGION 1..14: note = PR300526 HFR2
  source 1..14: note = PR300526 HFR2
WVRQAPGQGLEWMG

SEQ ID NO: 7 - protein, 17 aa, synthetic construct
  REGION 1..17: note = PR300526 HCDR2
  source 1..17: note = PR300526 HCDR2
WINPNSDGTNYAQRFQG

SEQ ID NO: 8 - protein, 32 aa, synthetic construct
  REGION 1..32: note = PR300526 HFR3
  source 1..32: note = PR300526 HFR3
RVTMTRDTSISTAYMELSRLRSDDTAVYYCAR

SEQ ID NO: 9 - protein, 15 aa, synthetic construct
  REGION 1..15: note = PR300526 HCDR3
  source 1..15: note = PR300526 HCDR3
GRLLRFFDWLDVMDA

SEQ ID NO: 10 - protein, 11 aa, synthetic construct
  REGION 1..11: note = PR300526 HFR4
  source 1..11: note = PR300526 HFR4
WGQGTSVTVSS

SEQ ID NO: 11 - protein, 220 aa, synthetic construct
  REGION 1..220: note = PR300526 L
  source 1..220: note = PR300526 L
DIVMTQSPDSLAVSLGERATINCKSSRSVLYSSNNKNYLAWYQQKPGQPPKLLIYWASTRESGVPDRFSGSGSGTDFTLTISSLQAEDVAVYYCQQYYSIPYTFGQGTKLEIKRTVAAPSVFIFPPSDEQLKSGTASVVCLLNNFYPREAKVQWKVDNALQSGNSQESVTEQDSKDSTYSLSSTLTLSKADYEKHKVYACEVTHQGLSSPVTKSFNRGEC

SEQ ID NO: 12 - protein, 113 aa, synthetic construct
  REGION 1..113: note = PR300526 VL
  source 1..113: note = PR300526 VL
DIVMTQSPDSLAVSLGERATINCKSSRSVLYSSNNKNYLAWYQQKPGQPPKLLIYWASTRESGVPDRFSGSGSGTDFTLTISSLQAEDVAVYYCQQYYSIPYTFGQGTKLEIK

SEQ ID NO: 13 - protein, 23 aa, synthetic construct
  REGION 1..23: note = PR300526 LFR1
  source 1..23: note = PR300526 LFR1
DIVMTQSPDSLAVSLGERATINC

SEQ ID NO: 14 - protein, 17 aa, synthetic construct
  REGION 1..17: note = PR300526 LCDR1
  source 1..17: note = PR300526 LCDR1
KSSRSVLYSSNNKNYLA

SEQ ID NO: 15 - protein, 15 aa, synthetic construct
  REGION 1..15: note = PR300526 LFR2
  source 1..15: note = PR300526 LFR2
WYQQKPGQPPKLLIY

SEQ ID NO: 16 - protein, 7 aa, synthetic construct
  REGION 1..7: note = PR300526 LCDR2
  source 1..7: note = PR300526 LCDR2
WASTRES

SEQ ID NO: 17 - protein, 32 aa, synthetic construct
  REGION 1..32: note = PR300526 LFR3
  source 1..32: note = PR300526 LFR3
GVPDRFSGSGSGTDFTLTISSLQAEDVAVYYC

SEQ ID NO: 18 - protein, 9 aa, synthetic construct
  REGION 1..9: note = PR300526 LCDR3
  source 1..9: note = PR300526 LCDR3
QQYYSIPYT

SEQ ID NO: 19 - protein, 10 aa, synthetic construct
  REGION 1..10: note = PR300526 LFR4
  source 1..10: note = PR300526 LFR4
FGQGTKLEIK

SEQ ID NO: 20 - protein, 458 aa, synthetic construct
  REGION 1..458: note = PR300659 H
  source 1..458: note = PR300659 H
QVQLVESGGGVVQPGRSLRLSCAASGFIFSSYDIYWVRQAPGKGLEWVAVIWHDGSNKYYADSVKGRFTISRDNSKNTVYLQMNSLRAEDTAVYYCARDTHSYGSRIYYDYNYGMDVWGQGTTVTVSSASTKGPSVFPLAPSSKSTSGGTAALGCLVKDYFPEPVTVSWNSGALTSGVHTFPAVLQSSGLYSLSSVVTVPSSSLGTQTYICNVNHKPSNTKVDKKVEPKSCDKTHTCPPCPAPELLGGPSVFLFPPKPKDTLMISRTPEVTCVVVDVSHEDPEVKFNWYVDGVEVHNAKTKPREEQYNSTYRVVSVLTVLHQDWLNGKEYKCKVSNKALPAPIEKTISKAKGQPREPQVYTLPPSREEMTKNQVSLTCLVKGFYPSDIAVEWESNGQPENNYKTTPPVLDSDGSFFLYSKLTVDKSRWQQGNVFSCSVMHEALHNHYTQKSLSLSPGK

SEQ ID NO: 21 - protein, 128 aa, synthetic construct
  REGION 1..128: note = PR300659 VH
  source 1..128: note = PR300659 VH
QVQLVESGGGVVQPGRSLRLSCAASGFIFSSYDIYWVRQAPGKGLEWVAVIWHDGSNKYYADSVKGRFTISRDNSKNTVYLQMNSLRAEDTAVYYCARDTHSYGSRIYYDYNYGMDVWGQGTTVTVSS

SEQ ID NO: 22 - protein, 25 aa, synthetic construct
  REGION 1..25: note = PR300659 HFR1
  source 1..25: note = PR300659 HFR1
QVQLVESGGGVVQPGRSLRLSCAAS

SEQ ID NO: 23 - protein, 10 aa, synthetic construct
  REGION 1..10: note = PR300659 HCDR1
  source 1..10: note = PR300659 HCDR1
GFIFSSYDIY

SEQ ID NO: 24 - protein, 14 aa, synthetic construct
  REGION 1..14: note = PR300659 HFR2
  source 1..14: note = PR300659 HFR2
WVRQAPGKGLEWVA

SEQ ID NO: 25 - protein, 17 aa, synthetic construct
  REGION 1..17: note = PR300659 HCDR2
  source 1..17: note = PR300659 HCDR2
VIWHDGSNKYYADSVKG

SEQ ID NO: 26 - protein, 32 aa, synthetic construct
  REGION 1..32: note = PR300659 HFR3
  source 1..32: note = PR300659 HFR3
RFTISRDNSKNTVYLQMNSLRAEDTAVYYCAR

SEQ ID NO: 27 - protein, 19 aa, synthetic construct
  REGION 1..19: note = PR300659 HCDR3
  source 1..19: note = PR300659 HCDR3
DTHSYGSRIYYDYNYGMDV

SEQ ID NO: 28 - protein, 11 aa, synthetic construct
  REGION 1..11: note = PR300659 HFR4
  source 1..11: note = PR300659 HFR4
WGQGTTVTVSS

SEQ ID NO: 29 - protein, 214 aa, synthetic construct
  REGION 1..214: note = PR300659 L
  source 1..214: note = PR300659 L
DIQMTQSPSSLSASVGDRVSITCRASQSISSYLNWYQQKPGKAPKLLIYAASSLQSGVPSRFSGSGSGADFTLTISSLQPEDFATYYCQQTYSPPFTFGPGTKVDIKRTVAAPSVFIFPPSDEQLKSGTASVVCLLNNFYPREAKVQWKVDNALQSGNSQESVTEQDSKDSTYSLSSTLTLSKADYEKHKVYACEVTHQGLSSPVTKSFNRGEC

SEQ ID NO: 30 - protein, 107 aa, synthetic construct
  REGION 1..107: note = PR300659 VL
  source 1..107: note = PR300659 VL
DIQMTQSPSSLSASVGDRVSITCRASQSISSYLNWYQQKPGKAPKLLIYAASSLQSGVPSRFSGSGSGADFTLTISSLQPEDFATYYCQQTYSPPFTFGPGTKVDIK

SEQ ID NO: 31 - protein, 23 aa, synthetic construct
  REGION 1..23: note = PR300659 LFR1
  source 1..23: note = PR300659 LFR1
DIQMTQSPSSLSASVGDRVSITC

SEQ ID NO: 32 - protein, 11 aa, synthetic construct
  REGION 1..11: note = PR300659 LCDR1
  source 1..11: note = PR300659 LCDR1
RASQSISSYLN

SEQ ID NO: 33 - protein, 15 aa, synthetic construct
  REGION 1..15: note = PR300659 LFR2
  source 1..15: note = PR300659 LFR2
WYQQKPGKAPKLLIY

SEQ ID NO: 34 - protein, 7 aa, synthetic construct
  REGION 1..7: note = PR300659 LCDR2
  source 1..7: note = PR300659 LCDR2
AASSLQS

SEQ ID NO: 35 - protein, 32 aa, synthetic construct
  REGION 1..32: note = PR300659 LFR3
  source 1..32: note = PR300659 LFR3
GVPSRFSGSGSGADFTLTISSLQPEDFATYYC

SEQ ID NO: 36 - protein, 9 aa, synthetic construct
  REGION 1..9: note = PR300659 LCDR3
  source 1..9: note = PR300659 LCDR3
QQTYSPPFT

SEQ ID NO: 37 - protein, 10 aa, synthetic construct
  REGION 1..10: note = PR300659 LFR4
  source 1..10: note = PR300659 LFR4
FGPGTKVDIK

SEQ ID NO: 38 - protein, 460 aa, synthetic construct
  REGION 1..460: note = PR300670 H
  source 1..460: note = PR300670 H
QVQLVESGGGVVQPGRSLRLSCVASGFTFSTYGIHWVRQAPGKGLDWVSVIWYDGSHKYYADSVQDRFTISRDNSKNTLYLQMNSLRAEDTAVYYCAREGMITMVRGVIIDYQYHGMDVWGQGTTVTVSSASTKGPSVFPLAPSSKSTSGGTAALGCLVKDYFPEPVTVSWNSGALTSGVHTFPAVLQSSGLYSLSSVVTVPSSSLGTQTYICNVNHKPSNTKVDKKVEPKSCDKTHTCPPCPAPELLGGPSVFLFPPKPKDTLMISRTPEVTCVVVDVSHEDPEVKFNWYVDGVEVHNAKTKPREEQYNSTYRVVSVLTVLHQDWLNGKEYKCKVSNKALPAPIEKTISKAKGQPREPQVYTLPPSREEMTKNQVSLTCLVKGFYPSDIAVEWESNGQPENNYKTTPPVLDSDGSFFLYSKLTVDKSRWQQGNVFSCSVMHEALHNHYTQKSLSLSPGK

SEQ ID NO: 39 - protein, 130 aa, synthetic construct
  REGION 1..130: note = PR300670 VH
  source 1..130: note = PR300670 VH
QVQLVESGGGVVQPGRSLRLSCVASGFTFSTYGIHWVRQAPGKGLDWVSVIWYDGSHKYYADSVQDRFTISRDNSKNTLYLQMNSLRAEDTAVYYCAREGMITMVRGVIIDYQYHGMDVWGQGTTVTVSS

SEQ ID NO: 40 - protein, 25 aa, synthetic construct
  REGION 1..25: note = PR300670 HFR1
  source 1..25: note = PR300670 HFR1
QVQLVESGGGVVQPGRSLRLSCVAS

SEQ ID NO: 41 - protein, 10 aa, synthetic construct
  REGION 1..10: note = PR300670 HCDR1
  source 1..10: note = PR300670 HCDR1
GFTFSTYGIH

SEQ ID NO: 42 - protein, 14 aa, synthetic construct
  REGION 1..14: note = PR300670 HFR2
  source 1..14: note = PR300670 HFR2
WVRQAPGKGLDWVS

SEQ ID NO: 43 - protein, 17 aa, synthetic construct
  REGION 1..17: note = PR300670 HCDR2
  source 1..17: note = PR300670 HCDR2
VIWYDGSHKYYADSVQD

SEQ ID NO: 44 - protein, 32 aa, synthetic construct
  REGION 1..32: note = PR300670 HFR3
  source 1..32: note = PR300670 HFR3
RFTISRDNSKNTLYLQMNSLRAEDTAVYYCAR

SEQ ID NO: 45 - protein, 21 aa, synthetic construct
  REGION 1..21: note = PR300670 HCDR3
  source 1..21: note = PR300670 HCDR3
EGMITMVRGVIIDYQYHGMDV

SEQ ID NO: 46 - protein, 11 aa, synthetic construct
  REGION 1..11: note = PR300670 HFR4
  source 1..11: note = PR300670 HFR4
WGQGTTVTVSS

SEQ ID NO: 47 - protein, 214 aa, synthetic construct
  REGION 1..214: note = PR300670 L
  source 1..214: note = PR300670 L
DIQMTQSPSTLSASVGDRVTITCRASQSIGRRLAWYQQKPGKAPKLLIYKASSLESGVPSRFSGSGSGTEFTLTISSPQPDDFATYYCQQYHSYSYTFGQGTKLEIKRTVAAPSVFIFPPSDEQLKSGTASVVCLLNNFYPREAKVQWKVDNALQSGNSQESVTEQDSKDSTYSLSSTLTLSKADYEKHKVYACEVTHQGLSSPVTKSFNRGEC

SEQ ID NO: 48 - protein, 107 aa, synthetic construct
  REGION 1..107: note = PR300670 VL
  source 1..107: note = PR300670 VL
DIQMTQSPSTLSASVGDRVTITCRASQSIGRRLAWYQQKPGKAPKLLIYKASSLESGVPSRFSGSGSGTEFTLTISSPQPDDFATYYCQQYHSYSYTFGQGTKLEIK

SEQ ID NO: 49 - protein, 23 aa, synthetic construct
  REGION 1..23: note = PR300670 LFR1
  source 1..23: note = PR300670 LFR1
DIQMTQSPSTLSASVGDRVTITC

SEQ ID NO: 50 - protein, 11 aa, synthetic construct
  REGION 1..11: note = PR300670 LCDR1
  source 1..11: note = PR300670 LCDR1
RASQSIGRRLA

SEQ ID NO: 51 - protein, 15 aa, synthetic construct
  REGION 1..15: note = PR300670 LFR2
  source 1..15: note = PR300670 LFR2
WYQQKPGKAPKLLIY

SEQ ID NO: 52 - protein, 7 aa, synthetic construct
  REGION 1..7: note = PR300670 LCDR2
  source 1..7: note = PR300670 LCDR2
KASSLES

SEQ ID NO: 53 - protein, 32 aa, synthetic construct
  REGION 1..32: note = PR300670 LFR3
  source 1..32: note = PR300670 LFR3
GVPSRFSGSGSGTEFTLTISSPQPDDFATYYC

SEQ ID NO: 54 - protein, 9 aa, synthetic construct
  REGION 1..9: note = PR300670 LCDR3
  source 1..9: note = PR300670 LCDR3
QQYHSYSYT

SEQ ID NO: 55 - protein, 10 aa, synthetic construct
  REGION 1..10: note = PR300670 LFR4
  source 1..10: note = PR300670 LFR4
FGQGTKLEIK

SEQ ID NO: 56 - protein, 451 aa, synthetic construct
  REGION 1..451: note = PR300679 H
  source 1..451: note = PR300679 H
QVQLQESGPGLVKPSGTLSLTCAVSGGSISSSNWWSWVRQPPGKGLEWIGEIYHSGSTNYNPSLKSRVTISVDKSKNQFSLKLSSVTAADTAVYYCAREYSSSWLSVMDAWGQGASVTVSSASTKGPSVFPLAPSSKSTSGGTAALGCLVKDYFPEPVTVSWNSGALTSGVHTFPAVLQSSGLYSLSSVVTVPSSSLGTQTYICNVNHKPSNTKVDKKVEPKSCDKTHTCPPCPAPELLGGPSVFLFPPKPKDTLMISRTPEVTCVVVDVSHEDPEVKFNWYVDGVEVHNAKTKPREEQYNSTYRVVSVLTVLHQDWLNGKEYKCKVSNKALPAPIEKTISKAKGQPREPQVYTLPPSREEMTKNQVSLTCLVKGFYPSDIAVEWESNGQPENNYKTTPPVLDSDGSFFLYSKLTVDKSRWQQGNVFSCSVMHEALHNHYTQKSLSLSPGK

SEQ ID NO: 57 - protein, 121 aa, synthetic construct
  REGION 1..121: note = PR300679 VH
  source 1..121: note = PR300679 VH
QVQLQESGPGLVKPSGTLSLTCAVSGGSISSSNWWSWVRQPPGKGLEWIGEIYHSGSTNYNPSLKSRVTISVDKSKNQFSLKLSSVTAADTAVYYCAREYSSSWLSVMDAWGQGASVTVSS

SEQ ID NO: 58 - protein, 25 aa, synthetic construct
  REGION 1..25: note = PR300679 HFR1
  source 1..25: note = PR300679 HFR1
QVQLQESGPGLVKPSGTLSLTCAVS

SEQ ID NO: 59 - protein, 11 aa, synthetic construct
  REGION 1..11: note = PR300679 HCDR1
  source 1..11: note = PR300679 HCDR1
GGSISSSNWWS

SEQ ID NO: 60 - protein, 14 aa, synthetic construct
  REGION 1..14: note = PR300679 HFR2
  source 1..14: note = PR300679 HFR2
WVRQPPGKGLEWIG

SEQ ID NO: 61 - protein, 16 aa, synthetic construct
  REGION 1..16: note = PR300679 HCDR2
  source 1..16: note = PR300679 HCDR2
EIYHSGSTNYNPSLKS

SEQ ID NO: 62 - protein, 32 aa, synthetic construct
  REGION 1..32: note = PR300679 HFR3
  source 1..32: note = PR300679 HFR3
RVTISVDKSKNQFSLKLSSVTAADTAVYYCAR

SEQ ID NO: 63 - protein, 12 aa, synthetic construct
  REGION 1..12: note = PR300679 HCDR3
  source 1..12: note = PR300679 HCDR3
EYSSSWLSVMDA

SEQ ID NO: 64 - protein, 11 aa, synthetic construct
  REGION 1..11: note = PR300679 HFR4
  source 1..11: note = PR300679 HFR4
WGQGASVTVSS

SEQ ID NO: 65 - protein, 215 aa, synthetic construct
  REGION 1..215: note = PR300679 L
  source 1..215: note = PR300679 L
EIVLTQSPGTLSLSPGERATLSCRASQSVSSSYLAWYQQKPGQAPRLLIYGASSRATGIPDRFSGSGSGTDFTLTISRLEPEDFAVYYCQQYGSSPRTFGQGTKVEIKRTVAAPSVFIFPPSDEQLKSGTASVVCLLNNFYPREAKVQWKVDNALQSGNSQESVTEQDSKDSTYSLSSTLTLSKADYEKHKVYACEVTHQGLSSPVTKSFNRGEC

SEQ ID NO: 66 - protein, 108 aa, synthetic construct
  REGION 1..108: note = PR300679 VL
  source 1..108: note = PR300679 VL
EIVLTQSPGTLSLSPGERATLSCRASQSVSSSYLAWYQQKPGQAPRLLIYGASSRATGIPDRFSGSGSGTDFTLTISRLEPEDFAVYYCQQYGSSPRTFGQGTKVEIK

SEQ ID NO: 67 - protein, 23 aa, synthetic construct
  REGION 1..23: note = PR300679 LFR1
  source 1..23: note = PR300679 LFR1
EIVLTQSPGTLSLSPGERATLSC

SEQ ID NO: 68 - protein, 12 aa, synthetic construct
  REGION 1..12: note = PR300679 LCDR1
  source 1..12: note = PR300679 LCDR1
RASQSVSSSYLA

SEQ ID NO: 69 - protein, 15 aa, synthetic construct
  REGION 1..15: note = PR300679 LFR2
  source 1..15: note = PR300679 LFR2
WYQQKPGQAPRLLIY

SEQ ID NO: 70 - protein, 7 aa, synthetic construct
  REGION 1..7: note = PR300679 LCDR2
  source 1..7: note = PR300679 LCDR2
GASSRAT

SEQ ID NO: 71 - protein, 32 aa, synthetic construct
  REGION 1..32: note = PR300679 LFR3
  source 1..32: note = PR300679 LFR3
GIPDRFSGSGSGTDFTLTISRLEPEDFAVYYC

SEQ ID NO: 72 - protein, 9 aa, synthetic construct
  REGION 1..9: note = PR300679 LCDR3
  source 1..9: note = PR300679 LCDR3
QQYGSSPRT

SEQ ID NO: 73 - protein, 10 aa, synthetic construct
  REGION 1..10: note = PR300679 LFR4
  source 1..10: note = PR300679 LFR4
FGQGTKVEIK

SEQ ID NO: 74 - protein, 449 aa, synthetic construct
  REGION 1..449: note = PR301285 H
  source 1..449: note = PR301285 H
QVQLQESGPGLVKPSETLSLTCTVSGGSMISYYWSWLRQPPGKGLEWIGYIYYSGNTNYNPSLKSRITIAVDTSKNQFSLKLNSVTAADTAVYYCARERELHPYYFDYWGQGTLVTVSSASTKGPSVFPLAPSSKSTSGGTAALGCLVKDYFPEPVTVSWNSGALTSGVHTFPAVLQSSGLYSLSSVVTVPSSSLGTQTYICNVNHKPSNTKVDKKVEPKSCDKTHTCPPCPAPELLGGPSVFLFPPKPKDTLMISRTPEVTCVVVDVSHEDPEVKFNWYVDGVEVHNAKTKPREEQYNSTYRVVSVLTVLHQDWLNGKEYKCKVSNKALPAPIEKTISKAKGQPREPQVYTLPPSREEMTKNQVSLTCLVKGFYPSDIAVEWESNGQPENNYKTTPPVLDSDGSFFLYSKLTVDKSRWQQGNVFSCSVMHEALHNHYTQKSLSLSPGK

SEQ ID NO: 75 - protein, 119 aa, synthetic construct
  REGION 1..119: note = PR301285 VH
  source 1..119: note = PR301285 VH
QVQLQESGPGLVKPSETLSLTCTVSGGSMISYYWSWLRQPPGKGLEWIGYIYYSGNTNYNPSLKSRITIAVDTSKNQFSLKLNSVTAADTAVYYCARERELHPYYFDYWGQGTLVTVSS

SEQ ID NO: 76 - protein, 25 aa, synthetic construct
  REGION 1..25: note = PR301285 HFR1
  source 1..25: note = PR301285 HFR1
QVQLQESGPGLVKPSETLSLTCTVS

SEQ ID NO: 77 - protein, 10 aa, synthetic construct
  REGION 1..10: note = PR301285 HCDR1
  source 1..10: note = PR301285 HCDR1
GGSMISYYWS

SEQ ID NO: 78 - protein, 14 aa, synthetic construct
  REGION 1..14: note = PR301285 HFR2
  source 1..14: note = PR301285 HFR2
WLRQPPGKGLEWIG

SEQ ID NO: 79 - protein, 16 aa, synthetic construct
  REGION 1..16: note = PR301285 HCDR2
  source 1..16: note = PR301285 HCDR2
YIYYSGNTNYNPSLKS

SEQ ID NO: 80 - protein, 32 aa, synthetic construct
  REGION 1..32: note = PR301285 HFR3
  source 1..32: note = PR301285 HFR3
RITIAVDTSKNQFSLKLNSVTAADTAVYYCAR

SEQ ID NO: 81 - protein, 11 aa, synthetic construct
  REGION 1..11: note = PR301285 HCDR3
  source 1..11: note = PR301285 HCDR3
ERELHPYYFDY

SEQ ID NO: 82 - protein, 11 aa, synthetic construct
  REGION 1..11: note = PR301285 HFR4
  source 1..11: note = PR301285 HFR4
WGQGTLVTVSS

SEQ ID NO: 83 - protein, 214 aa, synthetic construct
  REGION 1..214: note = PR301285 L
  source 1..214: note = PR301285 L
DIQLTQSPSFLSASVGDRVTITCRASQGIDNYLAWYQQKPGKAPKVLIYAASTLQSGVPSRFSGSGSGTEFTLTISSLQPEDFATYYCQQLNSYPLTFGGGTKVEIKRTVAAPSVFIFPPSDEQLKSGTASVVCLLNNFYPREAKVQWKVDNALQSGNSQESVTEQDSKDSTYSLSSTLTLSKADYEKHKVYACEVTHQGLSSPVTKSFNRGEC

SEQ ID NO: 84 - protein, 107 aa, synthetic construct
  REGION 1..107: note = PR301285 VL
  source 1..107: note = PR301285 VL
DIQLTQSPSFLSASVGDRVTITCRASQGIDNYLAWYQQKPGKAPKVLIYAASTLQSGVPSRFSGSGSGTEFTLTISSLQPEDFATYYCQQLNSYPLTFGGGTKVEIK

SEQ ID NO: 85 - protein, 23 aa, synthetic construct
  REGION 1..23: note = PR301285 LFR1
  source 1..23: note = PR301285 LFR1
DIQLTQSPSFLSASVGDRVTITC

SEQ ID NO: 86 - protein, 11 aa, synthetic construct
  REGION 1..11: note = PR301285 LCDR1
  source 1..11: note = PR301285 LCDR1
RASQGIDNYLA

SEQ ID NO: 87 - protein, 15 aa, synthetic construct
  REGION 1..15: note = PR301285 LFR2
  source 1..15: note = PR301285 LFR2
WYQQKPGKAPKVLIY

SEQ ID NO: 88 - protein, 7 aa, synthetic construct
  REGION 1..7: note = PR301285 LCDR2
  source 1..7: note = PR301285 LCDR2
AASTLQS

SEQ ID NO: 89 - protein, 32 aa, synthetic construct
  REGION 1..32: note = PR301285 LFR3
  source 1..32: note = PR301285 LFR3
GVPSRFSGSGSGTEFTLTISSLQPEDFATYYC

SEQ ID NO: 90 - protein, 9 aa, synthetic construct
  REGION 1..9: note = PR301285 LCDR3
  source 1..9: note = PR301285 LCDR3
QQLNSYPLT

SEQ ID NO: 91 - protein, 10 aa, synthetic construct
  REGION 1..10: note = PR301285 LFR4
  source 1..10: note = PR301285 LFR4
FGGGTKVEIK

SEQ ID NO: 92 - protein, 450 aa, synthetic construct
  REGION 1..450: note = PR301286 H
  source 1..450: note = PR301286 H
QVQLVESGGGVVQPGKSLRLSCAASGFTFSSYGMHWVRQAPGKGLEWVAVIWIDGSNRYYAASVKGRFTISRDNSKNTLYLQMNSLRAEDTAVYYCTRGYGDYAYVMDVWGQGASVTVSSASTKGPSVFPLAPSSKSTSGGTAALGCLVKDYFPEPVTVSWNSGALTSGVHTFPAVLQSSGLYSLSSVVTVPSSSLGTQTYICNVNHKPSNTKVDKKVEPKSCDKTHTCPPCPAPELLGGPSVFLFPPKPKDTLMISRTPEVTCVVVDVSHEDPEVKFNWYVDGVEVHNAKTKPREEQYNSTYRVVSVLTVLHQDWLNGKEYKCKVSNKALPAPIEKTISKAKGQPREPQVYTLPPSREEMTKNQVSLTCLVKGFYPSDIAVEWESNGQPENNYKTTPPVLDSDGSFFLYSKLTVDKSRWQQGNVFSCSVMHEALHNHYTQKSLSLSPGK

SEQ ID NO: 93 - protein, 120 aa, synthetic construct
  REGION 1..120: note = PR301286 VH
  source 1..120: note = PR301286 VH
QVQLVESGGGVVQPGKSLRLSCAASGFTFSSYGMHWVRQAPGKGLEWVAVIWIDGSNRYYAASVKGRFTISRDNSKNTLYLQMNSLRAEDTAVYYCTRGYGDYAYVMDVWGQGASVTVSS

SEQ ID NO: 94 - protein, 25 aa, synthetic construct
  REGION 1..25: note = PR301286 HFR1
  source 1..25: note = PR301286 HFR1
QVQLVESGGGVVQPGKSLRLSCAAS

SEQ ID NO: 95 - protein, 10 aa, synthetic construct
  REGION 1..10: note = PR301286 HCDR1
  source 1..10: note = PR301286 HCDR1
GFTFSSYGMH

SEQ ID NO: 96 - protein, 14 aa, synthetic construct
  REGION 1..14: note = PR301286 HFR2
  source 1..14: note = PR301286 HFR2
WVRQAPGKGLEWVA

SEQ ID NO: 97 - protein, 17 aa, synthetic construct
  REGION 1..17: note = PR301286 HCDR2
  source 1..17: note = PR301286 HCDR2
VIWIDGSNRYYAASVKG

SEQ ID NO: 98 - protein, 32 aa, synthetic construct
  REGION 1..32: note = PR301286 HFR3
  source 1..32: note = PR301286 HFR3
RFTISRDNSKNTLYLQMNSLRAEDTAVYYCTR

SEQ ID NO: 99 - protein, 11 aa, synthetic construct
  REGION 1..11: note = PR301286 HCDR3
  source 1..11: note = PR301286 HCDR3
GYGDYAYVMDV

SEQ ID NO: 100 - protein, 11 aa, synthetic construct
  REGION 1..11: note = PR301286 HFR4
  source 1..11: note = PR301286 HFR4
WGQGASVTVSS

SEQ ID NO: 101 - protein, 219 aa, synthetic construct
  REGION 1..219: note = PR301286 L
  source 1..219: note = PR301286 L
DIVMTQSPLSLPVTPGEPASISCRSSQSLLPGNGYNYLDWYLQKPGQSPQLLIYLGSNRASGVPDRFSGSGSGTDFTLKISRVEAEDVGIYYCMQALQSPLTFGGGTKVEIKRTVAAPSVFIFPPSDEQLKSGTASVVCLLNNFYPREAKVQWKVDNALQSGNSQESVTEQDSKDSTYSLSSTLTLSKADYEKHKVYACEVTHQGLSSPVTKSFNRGEC

SEQ ID NO: 102 - protein, 112 aa, synthetic construct
  REGION 1..112: note = PR301286 VL
  source 1..112: note = PR301286 VL
DIVMTQSPLSLPVTPGEPASISCRSSQSLLPGNGYNYLDWYLQKPGQSPQLLIYLGSNRASGVPDRFSGSGSGTDFTLKISRVEAEDVGIYYCMQALQSPLTFGGGTKVEIK

SEQ ID NO: 103 - protein, 23 aa, synthetic construct
  REGION 1..23: note = PR301286 LFR1
  source 1..23: note = PR301286 LFR1
DIVMTQSPLSLPVTPGEPASISC

SEQ ID NO: 104 - protein, 16 aa, synthetic construct
  REGION 1..16: note = PR301286 LCDR1
  source 1..16: note = PR301286 LCDR1
RSSQSLLPGNGYNYLD

SEQ ID NO: 105 - protein, 15 aa, synthetic construct
  REGION 1..15: note = PR301286 LFR2
  source 1..15: note = PR301286 LFR2
WYLQKPGQSPQLLIY

SEQ ID NO: 106 - protein, 7 aa, synthetic construct
  REGION 1..7: note = PR301286 LCDR2
  source 1..7: note = PR301286 LCDR2
LGSNRAS

SEQ ID NO: 107 - protein, 32 aa, synthetic construct
  REGION 1..32: note = PR301286 LFR3
  source 1..32: note = PR301286 LFR3
GVPDRFSGSGSGTDFTLKISRVEAEDVGIYYC

SEQ ID NO: 108 - protein, 9 aa, synthetic construct
  REGION 1..9: note = PR301286 LCDR3
  source 1..9: note = PR301286 LCDR3
MQALQSPLT

SEQ ID NO: 109 - protein, 10 aa, synthetic construct
  REGION 1..10: note = PR301286 LFR4
  source 1..10: note = PR301286 LFR4
FGGGTKVEIK

SEQ ID NO: 110 - protein, 450 aa, synthetic construct
  REGION 1..450: note = PR301286-1 H
  source 1..450: note = PR301286-1 H
QVQLVESGGGVVQPGKSLRLSCAASGFTFSSYGMHWVRQAPGKGLEWVAVIWIDASNRYYAASVKGRFTISRDNSKNTLYLQMNSLRAEDTAVYYCTRGYGDYAYVMDVWGQGASVTVSSASTKGPSVFPLAPSSKSTSGGTAALGCLVKDYFPEPVTVSWNSGALTSGVHTFPAVLQSSGLYSLSSVVTVPSSSLGTQTYICNVNHKPSNTKVDKKVEPKSCDKTHTCPPCPAPELLGGPSVFLFPPKPKDTLMISRTPEVTCVVVDVSHEDPEVKFNWYVDGVEVHNAKTKPREEQYNSTYRVVSVLTVLHQDWLNGKEYKCKVSNKALPAPIEKTISKAKGQPREPQVYTLPPSREEMTKNQVSLTCLVKGFYPSDIAVEWESNGQPENNYKTTPPVLDSDGSFFLYSKLTVDKSRWQQGNVFSCSVMHEALHNHYTQKSLSLSPGK

SEQ ID NO: 111 - protein, 120 aa, synthetic construct
  REGION 1..120: note = PR301286-1 VH
  source 1..120: note = PR301286-1 VH
QVQLVESGGGVVQPGKSLRLSCAASGFTFSSYGMHWVRQAPGKGLEWVAVIWIDASNRYYAASVKGRFTISRDNSKNTLYLQMNSLRAEDTAVYYCTRGYGDYAYVMDVWGQGASVTVSS

SEQ ID NO: 112 - protein, 17 aa, synthetic construct
  REGION 1..17: note = PR301286-1 HCDR2
  source 1..17: note = PR301286-1 HCDR2
VIWIDASNRYYAASVKG

SEQ ID NO: 113 - protein, 450 aa, synthetic construct
  REGION 1..450: note = PR301286-3 H
  source 1..450: note = PR301286-3 H
QVQLVESGGGVVQPGKSLRLSCAASGFTFSSYGMHWVRQAPGKGLEWVAVIWIDVSNRYYAASVKGRFTISRDNSKNTLYLQMNSLRAEDTAVYYCTRGYGDYAYVMDVWGQGASVTVSSASTKGPSVFPLAPSSKSTSGGTAALGCLVKDYFPEPVTVSWNSGALTSGVHTFPAVLQSSGLYSLSSVVTVPSSSLGTQTYICNVNHKPSNTKVDKKVEPKSCDKTHTCPPCPAPELLGGPSVFLFPPKPKDTLMISRTPEVTCVVVDVSHEDPEVKFNWYVDGVEVHNAKTKPREEQYNSTYRVVSVLTVLHQDWLNGKEYKCKVSNKALPAPIEKTISKAKGQPREPQVYTLPPSREEMTKNQVSLTCLVKGFYPSDIAVEWESNGQPENNYKTTPPVLDSDGSFFLYSKLTVDKSRWQQGNVFSCSVMHEALHNHYTQKSLSLSPGK

SEQ ID NO: 114 - protein, 120 aa, synthetic construct
  REGION 1..120: note = PR301286-3 VH
  source 1..120: note = PR301286-3 VH
QVQLVESGGGVVQPGKSLRLSCAASGFTFSSYGMHWVRQAPGKGLEWVAVIWIDVSNRYYAASVKGRFTISRDNSKNTLYLQMNSLRAEDTAVYYCTRGYGDYAYVMDVWGQGASVTVSS

SEQ ID NO: 115 - protein, 17 aa, synthetic construct
  REGION 1..17: note = PR301286-3 HCDR2
  source 1..17: note = PR301286-3 HCDR2
VIWIDVSNRYYAASVKG

SEQ ID NO: 116 - protein, 450 aa, synthetic construct; identical to SEQ ID NO: 110
  REGION 1..450: note = PR301286-5 PR301286-6 PR301286-7 H
  source 1..450: note = PR301286-5 PR301286-6 PR301286-7 H

SEQ ID NO: 117 - protein, 120 aa, synthetic construct; identical to SEQ ID NO: 111
  REGION 1..120: note = PR301286-5 PR301286-6 PR301286-7 VH
  source 1..120: note = PR301286-5 PR301286-6 PR301286-7 VH

SEQ ID NO: 118 - protein, 17 aa, synthetic construct
  REGION 1..17: note = PR301286-5 PR301286-6 PR301286-7 HCDR2
  source 1..17: note = PR301286-5 PR301286-6 PR301286-7 HCDR2
VIWIDASNRYYAASVKG

SEQ ID NO: 119 - protein, 219 aa, synthetic construct
  REGION 1..219: note = PR301286-5 L
  source 1..219: note = PR301286-5 L
DIVMTQSPLSLPVTPGEPASISCRSSQSLLPGSGYNYLDWYLQKPGQSPQLLIYLGSNRASGVPDRFSGSGSGTDFTLKISRVEAEDVGIYYCMQALQSPLTFGGGTKVEIKRTVAAPSVFIFPPSDEQLKSGTASVVCLLNNFYPREAKVQWKVDNALQSGNSQESVTEQDSKDSTYSLSSTLTLSKADYEKHKVYACEVTHQGLSSPVTKSFNRGEC

SEQ ID NO: 120 - protein, 112 aa, synthetic construct
  REGION 1..112: note = PR301286-5 VL
  source 1..112: note = PR301286-5 VL
DIVMTQSPLSLPVTPGEPASISCRSSQSLLPGSGYNYLDWYLQKPGQSPQLLIYLGSNRASGVPDRFSGSGSGTDFTLKISRVEAEDVGIYYCMQALQSPLTFGGGTKVEIK

SEQ ID NO: 121 - protein, 16 aa, synthetic construct
  REGION 1..16: note = PR301286-5 LCDR1
  source 1..16: note = PR301286-5 LCDR1
RSSQSLLPGSGYNYLD

SEQ ID NO: 122 - protein, 219 aa, synthetic construct
  REGION 1..219: note = PR301286-6 L
  source 1..219: note = PR301286-6 L
DIVMTQSPLSLPVTPGEPASISCRSSQSLLPGNAYNYLDWYLQKPGQSPQLLIYLGSNRASGVPDRFSGSGSGTDFTLKISRVEAEDVGIYYCMQALQSPLTFGGGTKVEIKRTVAAPSVFIFPPSDEQLKSGTASVVCLLNNFYPREAKVQWKVDNALQSGNSQESVTEQDSKDSTYSLSSTLTLSKADYEKHKVYACEVTHQGLSSPVTKSFNRGEC

SEQ ID NO: 123 - protein, 112 aa, synthetic construct
  REGION 1..112: note = PR301286-6 VL
  source 1..112: note = PR301286-6 VL
DIVMTQSPLSLPVTPGEPASISCRSSQSLLPGNAYNYLDWYLQKPGQSPQLLIYLGSNRASGVPDRFSGSGSGTDFTLKISRVEAEDVGIYYCMQALQSPLTFGGGTKVEIK

SEQ ID NO: 124 - protein, 16 aa, synthetic construct
  REGION 1..16: note = PR301286-6 LCDR1
  source 1..16: note = PR301286-6 LCDR1
RSSQSLLPGNAYNYLD

SEQ ID NO: 125 - protein, 219 aa, synthetic construct
  REGION 1..219: note = PR301286-7 L
  source 1..219: note = PR301286-7 L
DIVMTQSPLSLPVTPGEPASISCRSSQSLLPGNTYNYLDWYLQKPGQSPQLLIYLGSNRASGVPDRFSGSGSGTDFTLKISRVEAEDVGIYYCMQALQSPLTFGGGTKVEIKRTVAAPSVFIFPPSDEQLKSGTASVVCLLNNFYPREAKVQWKVDNALQSGNSQESVTEQDSKDSTYSLSSTLTLSKADYEKHKVYACEVTHQGLSSPVTKSFNRGEC

SEQ ID NO: 126 - protein, 112 aa, synthetic construct
  REGION 1..112: note = PR301286-7 VL
  source 1..112: note = PR301286-7 VL
DIVMTQSPLSLPVTPGEPASISCRSSQSLLPGNTYNYLDWYLQKPGQSPQLLIYLGSNRASGVPDRFSGSGSGTDFTLKISRVEAEDVGIYYCMQALQSPLTFGGGTKVEIK

SEQ ID NO: 127 - protein, 16 aa, synthetic construct
  REGION 1..16: note = PR301286-7 LCDR1
  source 1..16: note = PR301286-7 LCDR1
RSSQSLLPGNTYNYLD

SEQ ID NO: 128 - protein, 451 aa, synthetic construct
  REGION 1..451: note = PR301289 H
  source 1..451: note = PR301289 H
QVQLVQSGAEVKKPGASVKVSCRASGYTFTSYDINWVRQATGQGLEWMGWMNPHSGDTGYAQNFQGRVTMTWNTSISTAYMELSSLRSEDTAVYYCARRRVGVYYYGMDVWGQGTTVTVSSASTKGPSVFPLAPSSKSTSGGTAALGCLVKDYFPEPVTVSWNSGALTSGVHTFPAVLQSSGLYSLSSVVTVPSSSLGTQTYICNVNHKPSNTKVDKKVEPKSCDKTHTCPPCPAPELLGGPSVFLFPPKPKDTLMISRTPEVTCVVVDVSHEDPEVKFNWYVDGVEVHNAKTKPREEQYNSTYRVVSVLTVLHQDWLNGKEYKCKVSNKALPAPIEKTISKAKGQPREPQVYTLPPSREEMTKNQVSLTCLVKGFYPSDIAVEWESNGQPENNYKTTPPVLDSDGSFFLYSKLTVDKSRWQQGNVFSCSVMHEALHNHYTQKSLSLSPGK

SEQ ID NO: 129 - protein, 121 aa, synthetic construct
  REGION 1..121: note = PR301289 VH
  source 1..121: note = PR301289 VH
QVQLVQSGAEVKKPGASVKVSCRASGYTFTSYDINWVRQATGQGLEWMGWMNPHSGDTGYAQNFQGRVTMTWNTSISTAYMELSSLRSEDTAVYYCARRRVGVYYYGMDVWGQGTTVTVSS

SEQ ID NO: 130 - protein, 25 aa, synthetic construct
  REGION 1..25: note = PR301289 HFR1
  source 1..25: note = PR301289 HFR1
QVQLVQSGAEVKKPGASVKVSCRAS

SEQ ID NO: 131 - protein, 10 aa, synthetic construct
  REGION 1..10: note = PR301289 HCDR1
  source 1..10: note = PR301289 HCDR1
GYTFTSYDIN

SEQ ID NO: 132 - protein, 14 aa, synthetic construct
  REGION 1..14: note = PR301289 HFR2
  source 1..14: note = PR301289 HFR2
WVRQATGQGLEWMG

SEQ ID NO: 133 - protein, 17 aa, synthetic construct
  REGION 1..17: note = PR301289 HCDR2
  source 1..17: note = PR301289 HCDR2
WMNPHSGDTGYAQNFQG

SEQ ID NO: 134 - protein, 32 aa, synthetic construct
  REGION 1..32: note = PR301289 HFR3
  source 1..32: note = PR301289 HFR3
RVTMTWNTSISTAYMELSSLRSEDTAVYYCAR

SEQ ID NO: 135 - protein, 12 aa, synthetic construct
  REGION 1..12: note = PR301289 HCDR3
  source 1..12: note = PR301289 HCDR3
RRVGVYYYGMDV

SEQ ID NO: 136 - protein, 11 aa, synthetic construct
  REGION 1..11: note = PR301289 HFR4
  source 1..11: note = PR301289 HFR4
WGQGTTVTVSS

SEQ ID NO: 137 - protein, 215 aa, synthetic construct
  REGION 1..215: note = PR301289 L
  source 1..215: note = PR301289 L
ENVLTQSPGTLSLSPGERATLSCRASQSVSSSYFGWYQQKPGQAPRLLIYGASSRATGIPDRFSGSGSGTDFTLTISRLEPEDFAVYYCQQYGSSPITFGQGTRLEIKRTVAAPSVFIFPPSDEQLKSGTASVVCLLNNFYPREAKVQWKVDNALQSGNSQESVTEQDSKDSTYSLSSTLTLSKADYEKHKVYACEVTHQGLSSPVTKSFNRGEC

SEQ ID NO: 138 - protein, 108 aa, synthetic construct
  REGION 1..108: note = PR301289 VL
  source 1..108: note = PR301289 VL
ENVLTQSPGTLSLSPGERATLSCRASQSVSSSYFGWYQQKPGQAPRLLIYGASSRATGIPDRFSGSGSGTDFTLTISRLEPEDFAVYYCQQYGSSPITFGQGTRLEIK

SEQ ID NO: 139 - protein, 23 aa, synthetic construct
  REGION 1..23: note = PR301289 LFR1
  source 1..23: note = PR301289 LFR1
ENVLTQSPGTLSLSPGERATLSC

SEQ ID NO: 140 - protein, 12 aa, synthetic construct
  REGION 1..12: note = PR301289 LCDR1
  source 1..12: note = PR301289 LCDR1
RASQSVSSSYFG

SEQ ID NO: 141 - protein, 15 aa, synthetic construct
  REGION 1..15: note = PR301289 LFR2
  source 1..15: note = PR301289 LFR2
WYQQKPGQAPRLLIY

SEQ ID NO: 142 - protein, 7 aa, synthetic construct
  REGION 1..7: note = PR301289 LCDR2
  source 1..7: note = PR301289 LCDR2
GASSRAT

SEQ ID NO: 143 - protein, 32 aa, synthetic construct; identical to SEQ ID NO: 71
  REGION 1..32: note = PR301289 LFR3
  source 1..32: note = PR301289 LFR3

SEQ ID NO: 144 - protein, 9 aa, synthetic construct
  REGION 1..9: note = PR301289 LCDR3
  source 1..9: note = PR301289 LCDR3
QQYGSSPIT

SEQ ID NO: 145 - protein, 10 aa, synthetic construct
  REGION 1..10: note = PR301289 LFR4
  source 1..10: note = PR301289 LFR4
FGQGTRLEIK

SEQ ID NO: 146 - protein, 451 aa, synthetic construct
  REGION 1..451: note = PR301289-1 H
  source 1..451: note = PR301289-1 H
QVQLVQSGAEVKKPGASVKVSCRASGYTFTSYDINWVRQATGQGLEWMGWMNPHSGDTGYAQNFQGRVTMTWQTSISTAYMELSSLRSEDTAVYYCARRRVGVYYYGMDVWGQGTTVTVSSASTKGPSVFPLAPSSKSTSGGTAALGCLVKDYFPEPVTVSWNSGALTSGVHTFPAVLQSSGLYSLSSVVTVPSSSLGTQTYICNVNHKPSNTKVDKKVEPKSCDKTHTCPPCPAPELLGGPSVFLFPPKPKDTLMISRTPEVTCVVVDVSHEDPEVKFNWYVDGVEVHNAKTKPREEQYNSTYRVVSVLTVLHQDWLNGKEYKCKVSNKALPAPIEKTISKAKGQPREPQVYTLPPSREEMTKNQVSLTCLVKGFYPSDIAVEWESNGQPENNYKTTPPVLDSDGSFFLYSKLTVDKSRWQQGNVFSCSVMHEALHNHYTQKSLSLSPGK

SEQ ID NO: 147 - protein, 121 aa, synthetic construct
  REGION 1..121: note = PR301289-1 VH
  source 1..121: note = PR301289-1 VH
QVQLVQSGAEVKKPGASVKVSCRASGYTFTSYDINWVRQATGQGLEWMGWMNPHSGDTGYAQNFQGRVTMTWQTSISTAYMELSSLRSEDTAVYYCARRRVGVYYYGMDVWGQGTTVTVSS

SEQ ID NO: 148 - protein, 451 aa, synthetic construct
  REGION 1..451: note = PR301289-2 H
  source 1..451: note = PR301289-2 H
QVQLVQSGAEVKKPGASVKVSCRASGYTFTSYDINWVRQATGQGLEWMGWMNPHSGDTGYAQNFQGRVTMTWQTSISTAYMELSSLRSEDTAVYYCARRRVGVYYHGMDVWGQGTTVTVSSASTKGPSVFPLAPSSKSTSGGTAALGCLVKDYFPEPVTVSWNSGALTSGVHTFPAVLQSSGLYSLSSVVTVPSSSLGTQTYICNVNHKPSNTKVDKKVEPKSCDKTHTCPPCPAPELLGGPSVFLFPPKPKDTLMISRTPEVTCVVVDVSHEDPEVKFNWYVDGVEVHNAKTKPREEQYNSTYRVVSVLTVLHQDWLNGKEYKCKVSNKALPAPIEKTISKAKGQPREPQVYTLPPSREEMTKNQVSLTCLVKGFYPSDIAVEWESNGQPENNYKTTPPVLDSDGSFFLYSKLTVDKSRWQQGNVFSCSVMHEALHNHYTQKSLSLSPGK

SEQ ID NO: 149 - protein, 121 aa, synthetic construct
  REGION 1..121: note = PR301289-2 VH
  source 1..121: note = PR301289-2 VH
QVQLVQSGAEVKKPGASVKVSCRASGYTFTSYDINWVRQATGQGLEWMGWMNPHSGDTGYAQNFQGRVTMTWQTSISTAYMELSSLRSEDTAVYYCARRRVGVYYHGMDVWGQGTTVTVSS

SEQ ID NO: 150 - protein, 32 aa, synthetic construct
  REGION 1..32: note = PR301289-1 PR301289-2 HFR3
  source 1..32: note = PR301289-1 PR301289-2 HFR3
RVTMTWQTSISTAYMELSSLRSEDTAVYYCAR

SEQ ID NO: 151 - protein, 12 aa, synthetic construct
  REGION 1..12: note = PR301289-2 HCDR3
  source 1..12: note = PR301289-2 HCDR3
RRVGVYYHGMDV

SEQ ID NO: 152 - protein, 452 aa, synthetic construct
  REGION 1..452: note = PR300066(Tab) H
  source 1..452: note = PR300066(Tab) H
QVQLQQPGAELVKPGASVKMSCKASGYTFTSYWITWVIQRPGQGLEWIGDIYCGSDTMHYNEKFKNKATLTVDTSSSTAYMQLSSLTSEDSAVYYCARWWDYGSSYDYFDYWGQGTTLTVSSASTKGPSVFPLAPSSKSTSGGTAALGCLVKDYFPEPVTVSWNSGALTSGVHTFPAVLQSSGLYSLSSVVTVPSSSLGTQTYICNVNHKPSNTKVDKKVEPKSCDKTHTCPPCPAPELLGGPSVFLFPPKPKDTLMISRTPEVTCVVVDVSHEDPEVKFNWYVDGVEVHNAKTKPREEQYNSTYRVVSVLTVLHQDWLNGKEYKCKVSNKALPAPIEKTISKAKGQPREPQVYTLPPSREEMTKNQVSLTCLVKGFYPSDIAVEWESNGQPENNYKTTPPVLDSDGSFFLYSKLTVDKSRWQQGNVFSCSVMHEALHNHYTQKSLSLSPGK

SEQ ID NO: 153 - protein, 214 aa, synthetic construct
  REGION 1..214: note = PR300066(Tab) L
  source 1..214: note = PR300066(Tab) L
DIKMTQSPSSMYASLGERVTITCKASQDINSYLSWFQQKPGKSPKTLIYRANRLVDGVPSRFSGSGSGQDYSLTISSLEYEDMGIYYCLQYDEFPYTFGGGTKLEIKRTVAAPSVFIFPPSDEQLKSGTASVVCLLNNFYPREAKVQWKVDNALQSGNSQESVTEQDSKDSTYSLSSTLTLSKADYEKHKVYACEVTHQGLSSPVTKSFNRGEC

SEQ ID NO: 154 - protein, 482 aa, synthetic construct
  REGION 1..482: note = Recombined Siglec-15 ECD-hFc
  source 1..482: note = Recombined Siglec-15 ECD-hFc
FVRTKIDTTENLLNTEVHSSPAQRWSMQVPPEVSAEAGDAAVLPCTFTHPHRHYDGPLTAIWRAGEPYAGPQVFRCAAARGSELCQTALSLHGRFRLLGNPRRNDLSLRVERLALADDRRYFCRVEFAGDVHDRYESRHGVRLHVTAAPRIVNISVLPSPAHAFRALCTAEGEPPPALAWSGPALGNSLAAVRSPREGHGHLVTAELPALTHDGRYTCTAANSLGRSEASVYLFRFHGASGASTIEGRMDEPKSCDKTHTCPPCPAPELLGGPSVFLFPPKPKDTLMISRTPEVTCVVVDVSHEDPEVKFNWYVDGVEVHNAKTKPREEQYNSTYRVVSVLTVLHQDWLNGKEYKCKVSNKALPAPIEKTISKAKGQPREPQVYTLPPSRDELTKNQVSLTCLVKGFYPSDIAVEWESNGQPENNYKTTPPVLDSDGSFFLYSKLTVDKSRWQQGNVFSCSVMHEALHNHYTQKSLSLSPGK

SEQ ID NO: 155 - protein, 328 aa, Macaca fascicularis
MESSIRLLACLACVLPTGSFVRTKIDTTENLLNTEVHSSPAQRWSMQVPAEVSAAAGDAAVLPCTFTHPHRHYDGPLTAIWRAGEPYAGPQVFRCAAARGSELCQTALSLHGRFRLLGNPRRNDLSLRVERLALADDRRYFCRVEFAGDVHDRYESRHGVRLHVTAAPRIINISVLPGPAHAFRALCTAEGEPPPALAWSGPALGNGSAAVPSSGQGHGHLVTAELPALNHDGRYTCTAANSLGRSEASVYLFRFHGASGASTVALLLGALGLKALLLLGVLAAGVARRRPEHLNTPDTPPRSQAQESNYENLSQMNPRSPPAAMCSP

SEQ ID NO: 156 - protein, 240 aa, synthetic construct
  REGION 1..240: note = OS8
  source 1..240: note = OS8
QVQLQQSGAELARPGASVKMSCKASGYTFTRYTMHWVKQRPGQGLEWIGYINPSRGYTNYNQKFKDKATLTTDKSSSTAYMQLSSLTSEDSAVYYCARYYDDHYCLDYWGQGTTLTVSSGGGGSGGGGSGGGGSQIVLTQSPAIMSASPGEKVTMTCSASSSVSYMNWYQQKSGTSPKRWIYDTSKLASGVPAHFRGSGSGTSYSLTISGMEAEDAATYYCQQWSSNPFTFGSGTKLEIN